European Patent Application EP 4 491 182 A1, published January 15, 2025. Title: 四环类化合物在治疗肿瘤中的应用. Applicant: 南京施江医药科技有限公司. Application CN. The sequence listing filed with the application follows.

SEQUENCE LISTING (2 sequences)

SEQ ID NO: 1 - DNA, 2500 bp, synthetic construct
  source 1..2500: mol_type = other DNA
tatccaagagctatcagcactcccatgtttattgtagcactgttcacaatagccaagatttggaagtactctaagtgtccattagcagatgaatggataaagacaatgtggtaatacacataatggagtactattcagtcataaagaagaattagatcctgtcatttgcaataacatggatggaactggaggtcataatgttgagtgaaataaaccaggcacagaaagacaaactttgcatgttctcacttatttatgggagctaaaaactaaaataactgaactcacagagatagagagtagaaggatggttacgagaggatgggaagggtagcgaggtgggtaggggggatgtggggatcattaatgggtataaaaaatagttagaggccaggcgcagtggctcacgcctgtaatcccagcactttgggaggccgaggtaggcggaacacctgaggagttcaagaccagcctggccaatatgatgaaaccccgtctctactaaaaatacaaaaattagctgggcgtgatggtgtgcacctgtagtcccagctgcttgggaggctgaggcaggagaatcgctggaacccaagaggtgaaggttgcagtgagctgagatcgcgtcactgcactccagcctgggtgacagagtgagactccacatcaaaaaaaaaaaaaaaaagttagaaagattgaataagacctaatatttgctagcacaacagggtgaatatagtaaaaaataatttatttgtaccttcaaaaataactagacaagtataattgggttgtttgtaacacacaaaaaataagtacttgaagtggtggataccccatttaccctgatgtgattattttgtattgcaggcctctatcagaatatctcatgtaacccataaatatatacacctactctgtacccacaaaaagtttttaaaaagaaaaataaatagcaaccgaaaaaaaaagagagggagaaaagaaaaaagaaaaaaaaatcaagtgcctggctgggtagaataaattctaaggccacaatgttactgaccatgggttttttggctctcagtgtatagaaattgacacaaggccaatagtcttcccaaacatgctttactggaacttacgccctggcataagggccacaacaaaagagagagcgaattctctggcttgctgactccttggaaaaaaccggtagggatttttttattaggcaaagcacaggaattgacgtcagaggcaggatgtgctgctgggcaaagcatacgagaagtggggtatgcaggtcagcattacttggttgcaatggttatcttgaggaatgggccaactggtggtctggccagtggcaacaaggctgtaaatcaattattcagcattccttcccaaggtgggacacccggcaacattgtttatctcctaaggccagttcctggaattaagtgaaaggatgactaatggacatgttgtcagtgaggtagtggtgtgggttttgtgaccagtgggaatgcacgaaagaatgctttagcggggagtgagctgaagccaagccccatccctactctgtctcaaagtgagttcagaaaaggggatttaaagaattctttttttttttttttttttttttgagacagagtcttgctctgtcgcccaggctggagtgcagtggcgccatcttggctcactgcaagctccgccccccgggttcatgccattctcctgcctcagcctcccaagtagctgggactgcaggtgcctaccaccaagcccagctaattttttgtattttttttttagtagagacggggtttcaccatgttagccaggatggtctcgatctcctgacctcgtgatctgcccgccttagcctcccaaagtgctgggattacaggcatgagcctccgcccccggccttaaataattcttaaaggaagtaaagttaactttgaaagaactatcaggatttggattgactgaaaggagtggggaagcttagggaggaggtgcttgccagacactgggtcatggcagtggtcggtgaagctgcagttgcctagggcagggatggagagagagtctgggcatgaggagagggtctcgggatgtttggctggactagattttacagaaagccttatccaggcttttaaaattactctttccagacttcatctgagactccttcttcagccaacattccttagccctgaatacatttcctatcctcatctttcccttcttttttttcctttcttttacatgtttaaatttaaaccattcttcgtgaccccttttcttgggagattcatggcaagaacgagaagaatgatggtgcttgttaggggatgtcctgtctctctgaactttggggtcctatgcattaaataattttcctgacgagctcaagtgctccctctggtctacaatccctggcggctggccttcatcccttgggcaagcattgcatacagctcatggccctccctctaccataccc

SEQ ID NO: 2 - DNA, 64 bp, synthetic construct
  source 1..64: mol_type = other DNA
gatccgggatgagtccatcaaggaagattcaagagatcttccttgatggactcatccttttttg